European Patent Application EP 4 198 137 A1, published June 21, 2023. Title: Mischungen von Glucose und Xylose zur fermentativen Herstellung von ortho-Aminobenzoesäure. Applicant: Covestro Deutschland AG. The sequence listing filed with the application follows.

SEQUENCE LISTING (16 sequences)

SEQ ID NO: 1 - DNA, 1070 bp, artificial sequence
  Expressionskonstrukt
gccctgcaggtaaaaaaaggattgtgacttctccagcaacactgaaagttctcaacgcctacttggataaccccactccaaccctggaggaggcaattgaggtgttcaccccgctgaccgtgggtgaatacgatgacgtgcacatcgcagcgctgcttgccaccatccgtactcgcggtgagcagttcgctgatattgccggcgctgccaaggcgttcctcgcggcggctcgtccgttcccgattactggcgcaggtttgctagattccgctggtactggtggcgacggtgccaacaccatcaacatcaccaccggcgcatccctgatcgcagcatccggtggagtgaagctggttaagcacggcaaccgttcggtgagctccaagtccggctccgccgatgtgctggaagcgctgaatattcctttgggccttgatgtggatcgtgctgtgaagtggttcgaagcgtccaacttcaccttcctgttcgcacctgcgtacaaccctgcgattgcgcatgtgcagccggttcgccaggcgctgaaattccccaccatcttcaacacgcttggaccattgctgtccccggcgcgcccggagcgtcagatcatgggcgtggccaatgccaatcatggacagctcatcgccgaggtcttccgcgagttgggccgtacacgcgcgcttgttgtgcatggcgcaggcaccgatgagatcgcagtccacggcaccaccttggtgtgggagcttaaagaagacggcaccatcgagcattacaccatcgagcctgaggaccttggccttggccgctacacccttgaggatctcgtaggtggcctcggcactgagaacgccgaagctatgcgcgctactttcgcgggcaccggccctgatgcacaccgtgatgcgttggctgcgtccgcaggtgcgatgttctacctcaacggcgatgtcgactccttgaaagatggtgcacaaaaggcgctttccttgcttgccgacggcaccacccaggcatggttggccaagcacgaagagatcgattactcagaaaaggagtcttccaatgactag

SEQ ID NO: 2 - DNA, 1070 bp, artificial sequence
  Expressionskonstrukt
gccctgcaggtaaaaaaaggattttgacttctccagcaacactgaaagttctcaacgcctacttggataaccccactccaaccctggaggaggcaattgaggtgttcaccccgctgaccgtgggtgaatacgatgacgtgcacatcgcagcgctgcttgccaccatccgtactcgcggtgagcagttcgctgatattgccggcgctgccaaggcgttcctcgcggcggctcgtccgttcccgattactggcgcaggtttgctagattccgctggtactggtggcgacggtgccaacaccatcaacatcaccaccggcgcatccctgatcgcagcatccggtggagtgaagctggttaagcacggcaaccgttcggtgagctccaagtccggctccgccgatgtgctggaagcgctgaatattcctttgggccttgatgtggatcgtgctgtgaagtggttcgaagcgtccaacttcaccttcctgttcgcacctgcgtacaaccctgcgattgcgcatgtgcagccggttcgccaggcgctgaaattccccaccatcttcaacacgcttggaccattgctgtccccggcgcgcccggagcgtcagatcatgggcgtggccaatgccaatcatggacagctcatcgccgaggtcttccgcgagttgggccgtacacgcgcgcttgttgtgcatggcgcaggcaccgatgagatcgcagtccacggcaccaccttggtgtgggagcttaaagaagacggcaccatcgagcattacaccatcgagcctgaggaccttggccttggccgctacacccttgaggatctcgtaggtggcctcggcactgagaacgccgaagctatgcgcgctactttcgcgggcaccggccctgatgcacaccgtgatgcgttggctgcgtccgcaggtgcgatgttctacctcaacggcgatgtcgactccttgaaagatggtgcacaaaaggcgctttccttgcttgccgacggcaccacccaggcatggttggccaagcacgaagagatcgattactcagaaaaggagtcttccaatgactag

SEQ ID NO: 3 - protein, 348 aa, Corynebacterium glutamicum
MTSPATLKVLNAYLDNPTPTLEEAIEVFTPLTVGEYDDVHIAALLATIRTRGEQFADIAGAAKAFLAAARPFPITGAGLLDSAGTGGDGANTINITTGASLIAASGGVKLVKHGNRSVSSKSGSADVLEALNIPLGLDVDRAVKWFEASNFTFLFAPAYNPAIAHVQPVRQALKFPTIFNTLGPLLSPARPERQIMGVANANHGQLIAEVFRELGRTRALVVHGAGTDEIAVHGTTLVWELKEDGTIEHYTIEPEDLGLGRYTLEDLVGGLGTENAEAMRATFAGTGPDAHRDALAASAGAMFYLNGDVDSLKDGAQKALSLLADGTTQAWLAKHEEIDYSEKESSND

SEQ ID NO: 4 - protein, 919 aa, Corynebacterium glutamicum
MTDFLRDDIRFLGQILGEVIAEQEGQEVYELVEQARLTSFDIAKGNAEMDSLVQVFDGITPAKATPIARAFSHFALLANLAEDLYDEELREQALDAGDTPPDSTLDATWLKLNEGNVGAEAVADVLRNAEVAPVLTAHPTETRRRTVFDAQKWITTHMRERHALQSAEPTARTQSKLDEIEKNIRRRITILWQTALIRVARPRIEDEIEVGLRYYKLSLLEEIPRINRDVAVELRERFGEGVPLKPVVKPGSWIGGDHDGNPYVTAETVEYSTHRAAETVLKYYARQLHSLEHELSLSDRMNKVTPQLLALADAGHNDVPSRVDEPYRRAVHGVRGRILATTAELIGEDAVEGVWFKVFTPYASPEEFLNDALTIDHSLRESKDVLIADDRLSVLISAIESFGFNLYALDLRQNSESYEDVLTELFERAQVTANYRELSEAEKLEVLLKELRSPRPLIPHGSDEYSEVTDRELGIFRTASEAVKKFGPRMVPHCIISMASSVTDVLEPMVLLKEFGLIAANGDNPRGTVDVIPLFETIEDLQAGAGILDELWKIDLYRNYLLQRDNVQEVMLGYSDSNKDGGYFSANWALYDAELQLVELCRSAGVKLRLFHGRGGTVGRGGGPSYDAILAQPRGAVQGSVRITEQGEIISAKYGNPETARRNLEALVSATLEASLLDVSELTDHQRAYDIMSEISELSLKKYASLVHEDQGFIDYFTQSTPLQEIGSLNIGSRPSSRKQTSSVEDLRAIPWVLSWSQSRVMLPGWFGVGTALEQWIGEGEQATQRIAELQTLNESWPFFTSVLDNMAQVMSKAELRLAKLYADLIPDTEVAERVYSVIREEYFLTKKMFCVITGSDDLLDDNPLLARSVQRRYPYLLPLNVIQVEMMRRYRKGDQSEQVSRNIQLTMNGLSTALRNSG

SEQ ID NO: 5 - DNA, 2760 bp, Corynebacterium glutamicum
atgactgattttttacgcgatgacatcaggttcctcggtcaaatcctcggtgaggtaattgcggaacaagaaggccaggaggtttatgaactggtcgaacaagcgcgcctgacttcttttgatatcgccaagggcaacgccgaaatggatagcctggttcaggttttcgacggcattactccagccaaggcaacaccgattgctcgcgcattttcccacttcgctctgctggctaacctggcggaagacctctacgatgaagagcttcgtgaacaggctctcgatgcaggcgacacccctccggacagcactcttgatgccacctggctgaaactcaatgagggcaatgttggcgcagaagctgtggccgatgtgctgcgcaatgctgaggtggcgccggttctgactgcgcacccaactgagactcgccgccgcactgtttttgatgcgcaaaagtggatcaccacccacatgcgtgaacgccacgctttgcagtctgcggagcctaccgctcgtacgcaaagcaagttggatgagatcgagaagaacatccgccgtcgcatcaccattttgtggcagaccgcgttgattcgtgtggcccgcccacgtatcgaggacgagatcgaagtagggctgcgctactacaagctgagccttttggaagagattccacgtatcaaccgtgatgtggctgttgagcttcgtgagcgtttcggcgagggtgttcctttgaagcccgtggtcaagccaggttcctggattggtggagaccacgacggtaacccttatgtcaccgcggaaacagttgagtattccactcaccgcgctgcggaaaccgtgctcaagtactatgcacgccagctgcattccctcgagcatgagctcagcctgtcggaccgcatgaataaggtcaccccgcagctgcttgcgctggcagatgcagggcacaacgacgtgccaagccgcgtggatgagccttatcgacgcgccgtccatggcgttcgcggacgtatcctcgcgacgacggccgagctgatcggcgaggacgccgttgagggcgtgtggttcaaggtctttactccatacgcatctccggaagaattcttaaacgatgcgttgaccattgatcattctctgcgtgaatccaaggacgttctcattgccgatgatcgtttgtctgtgctgatttctgccatcgagagctttggattcaacctttacgcactggatctgcgccaaaactccgaaagctacgaggacgtcctcaccgagcttttcgaacgcgcccaagtcaccgcaaactaccgcgagctgtctgaagcagagaagcttgaggtgctgctgaaggaactgcgcagccctcgtccgctgatcccgcacggttcagatgaatacagcgaggtcaccgaccgcgagctcggcatcttccgcaccgcgtcggaggctgttaagaaattcgggccacggatggtgcctcactgcatcatctccatggcatcatcggtcaccgatgtgctcgagccgatggtgttgctcaaggaattcggactcatcgcagccaacggcgacaacccacgcggcaccgtcgatgtcatcccactgttcgaaaccatcgaagatctccaggccggcgccggaatcctcgacgaactgtggaaaattgatctctaccgcaactacctcctgcagcgcgacaacgtccaggaagtcatgctcggttactccgattccaacaaggatggcggatatttctccgcaaactgggcgctttacgacgcggaactgcagctcgtcgaactatgccgatcagccggggtcaagcttcgcctgttccacggccgtggtggcaccgtcggccgcggtggcggaccttcctacgacgcgattcttgcccagcccaggggggctgtccaaggttccgtgcgcatcaccgagcagggcgagatcatctccgctaagtacggcaaccccgaaaccgcgcgccgaaacctcgaagccctggtctcagccacgcttgaggcatcgcttctcgacgtctccgaactcaccgatcaccaacgcgcgtacgacatcatgagtgagatctctgagctcagcttgaagaagtacgcctccttggtgcacgaggatcaaggcttcatcgattacttcacccagtccacgccgctgcaggagattggatccctcaacatcggatccaggccttcctcacgcaagcagacctcctcggtggaagatttgcgagccatcccatgggtgctcagctggtcacagtctcgtgtcatgctgccaggctggtttggtgtcggaaccgcattagagcagtggattggcgaaggggagcaggccacccaacgcattgccgagctgcaaacactcaatgagtcctggccatttttcacctcagtgttggataacatggctcaggtgatgtccaaggcagagctgcgtttggcaaagctctacgcagacctgatcccagatacggaagtagccgagcgagtctattccgtcatccgcgaggagtacttcctgaccaagaagatgttctgcgtaatcaccggctctgatgatctgcttgatgacaacccacttctcgcacgctctgtccagcgccgatacccctacctgcttccactcaacgtgatccaggtagagatgatgcgacgctaccgaaaaggcgaccaaagcgagcaagtgtcccgcaacattcagctgaccatgaacggtctttccactgcgctgcgcaactccggctag

SEQ ID NO: 6 - protein, 185 aa, Corynebacterium glutamicum
MNDQIHLDHQSDDTSECSCPIVVLVGLPGAGKSTIGRRLARALNTELVDSDELIERATGKACGAVFSELGEPAFRELEAIHVAEALKSSGVVSLGGGSVLTESTRELLKGQDVVWIDVPVEEGIRRTANERSRPVLQAADPAEHYRNLVKVRTPLYEEVATYRLRTNNRSPQQVVAAVLHHLEID

SEQ ID NO: 7 - protein, 174 aa, Escherichia coli
MTQPLFLIGPRGCGKTTVGMALADSLNRRFVDTDQWLQSQLNMTVAEIVEREEWAGFRARETAALEAVTAPSTVIATGGGIILTEFNRHFMQNNGIVVYLCAPVSVLVNRLQAAPEEDLRPTLTGKPLSEEVQEVLEERDALYREVAHIIIDATNEPSQVISEIRSALAQTINC

SEQ ID NO: 8 - DNA, 179 bp, artificial sequence
  Pomotorsequenz
cacagggtagctggtagtttgaaaatcaacgccgttgcccttaggattcagtaactggcacattttgtaatgcgctagatctgtgtgctcagtcttccaggctgcttatcacagtgaaagcaaaaccaattcgtggctgcgaaagtcgtagccaccacgaagtccaggaggacatacat

SEQ ID NO: 9 - protein, 430 aa, Escherichia coli
MVFVSDSSISLPIWDAPRARGPIVSDLAIPGSKSITNRALILAALASTPSTIIDVLRSRDTDLMTDGLRSLGITITEEAVDRYRVEPGQLSAGSVECGLAGTVMRFLPPVAAFADGPVHFDGDPQARVRPMTSILDALRSLGVEVDNNNLPFTVNAGEVPEGGVVEIDASGSSQFVSGLLLSAPRFKNGVTVKHVGGRLPSMPHIEMTVDMLRSAGIEIEESENQWVVHPGEILGRTWRIEPDLSNATPFLAAAAVTGGTIKINHWPIKTTQPGDAIRSILERMGCEVELVAQGEGYDLSVTGPVALKGIEIDMSDIGELTPTVAALAALASTESRLTGIAHLRGHETDRLAALTAEINKLGGKCTELKDGLLIEPASLHGGVWHSYADHRMATAGAIIGLAVDGVQVEDIKTTSKTFPGFENVWEEMVG

SEQ ID NO: 10 - protein, 410 aa, Corynebacterium glutamicum
MLGMLRWTTAGESHGQALIATVEHMPAGVPVTKDEVSYQLARRRLGYGRGARMKFEQDALTFLTGIRHGLTLGSPISIMIGNTEWDKWTTIMSSDALDMEDPDNVAAMSSGRGAKLTRPRPGHADYAGMLKYGFDDARNVLERSSARETAARVAAATVARSFLRETLGVEVLSHVISIGASEPYTGAEPTFADIQAIDDSPVRAFGKDAEESMIAEIEAAKKAGDTLGGIVEVIVEGLPIGLGSHISGEDRLDAQIAAALMGIQAIKGVEIGDGFEEARRRGSEAHDEVFLDDNGVYRNTNRAGGLEGGMTNGETLRVRAGMKPISTVPRALKTIDMENGKAATGIHQRSDVCAVPAAGVVAEAMVTLVLARAVLQKFGGDSLSETKSNIDTYLKNIEERMKFEGLEDGA

SEQ ID NO: 11 - protein, 350 aa, artificial sequence
  modifiziertes Enzym
MNYQNDDLRIKEIKELLPPVALLEKFPATENAANTVAHARKAIHKILKGNDDRLLVVIGPCSIHDPVAAKEYATRVLALREELKDELEIVMRVYFEKPRTTVGWKGLINDPHMDNSFQINDGLRIARKLLLDINDSGLPAAGEFLDMITPQYLADLMSWGAIGARTTESQVHRELASGLSCPVGFKNGTDGTIKVAIDAINAAGAPHCFLFVTKWGHSAIVNTSGNGDCHIILRGGKEPNYSAKHVAEVKEGLNKAGLPAQVMIDFSHANSSKQFKKQMDVCADVCQQIAGGEKAIIGVMVESHLVEGNQSLESGEPLAYGKSITDACIGWEDTDALLRQLANAVKARRG

SEQ ID NO: 12 - protein, 446 aa, Xanthomonas campestris
MSNTVFIGAKEYFPGIGKIGFEGRDSDNPLAFKVYDANKQVAGKTMAEHLRFAVAYWHSFCGNGADPFGPGTRAYPWDVGNTALARAEAKSDAAFEFFTKLGVPYYCFHDIDLAPDADDIGEYENNLKHMVGIAKQRQADTGVKLLWGTANLFSHPRYMNGASTNPDFNVVARAAVQVKAAIDATVELGGENYVFWGGREGYACLHNTQMKREQDNMARFLTLARDYGRAIGFTGNFLIEPKPMEPMKHQYDFDSATVIGFLRQHGLDQDFKLNIEANHATLSGHSFEHDLQVASDAGLLGSIDANRGNPQNGWDTDQFPTDLYDTVGAMLVVLRQGGLAPGGLNFDAKVRRESSDPQDLFLAHIGGMDAFARGLEVANALLTSSPLETWRAQRYASFDSGAGADFANGTSTLADLAKYAAGKGEPTQVSGRQEAYENLINQYLTR

SEQ ID NO: 13 - protein, 463 aa, artificial sequence
  modifiziertes Enzym
MSNTVFIGAKEYFPGIGKIGFEGRDSDNPLAFKVYDANKQVAGKTMAEHLRFAVAYWHSFCGNGADPFGPGTRAYPWDVGNTALARAEAKSDAAFEFFTKLGVPYYCFHDIDLAPDADDIGEYENNLKHMVGIAKQRQADTGVKLLWGTANLFSHPRYMNGASTNPDFNVVARAAVQVKAAIDATVELGGENYVFWGGREGYACLHNTQMKREQDNMARFLTLARDYGRAIGFTGNFLIEPKPMEPMKHQYDFDSATVIGFLRQHGLDQDFKLNIEANHATLSGHSFEHDLQVASDAGLLGSIDANRGNPQNGWDTDQFPTDLYDTVGAMLVVLRQGGLAPGGLNFDAKVRRESSDPQDLFLAHIGGMDAFARGLEVANALLTSSPLETWRAQRYASFDSGAGADFANGTSTLADLAKYAAGKGEPTQVSGRQEAYENLINQYLTRHRVAGSLKINAVALRIQ

SEQ ID NO: 14 - protein, 460 aa, Corynebacterium glutamicum
MALVLGIDSSTQSCKALLVDAATGQVIDEGRASHPSGSEVDPRAWIAALDQATEGLLERADAVSIAGQQHGMVALDENDEIVRPALLWNDTRSAQAALDLNEEIGGDQAAVDATGSVYVASLTATKMRWMRDHEPENAARTASVMLPHDFLTWHLMGRGRKVTDHGDASGTGYYSTRDRAWRTDLAALALGHEVELPELLAPNAIAGTTPGGVKVAAGTGDNAAAALGLDLQPGDVSVSIGTSGVAGMTVQHSVHDPSGLVTGFADATGAYFPLACTLNGAPVLEFGRRILGVEWEEFDALALAAQPGSGGVTLQPYLEGERTPNRPAARGVLAGLNCATTREDFARATVEGLLLALDDAVTALVEATGVPVQRIQLIGGGARSQAVREIAPEIFGHEIVVPEPAEYVALGAARQAAWALSGEATPPQWPTPGSDPHRAPKNTELSTRYAKLRAATQGWY

SEQ ID NO: 15 - DNA, 3302 bp, artificial sequence
  Expressionskonstrukt
gatcccacagggtagctggtagtttgaaaatcaacgccgttgcccttaggattcagtaactggcacattttgtaatgcgctagatctgtgtgctcagtcttccaggctgcttatcacagtgaaagcaaaaccaattcgtggctgcgaaagtcgtagccaccacgaagtccaggaggacatacagtatgacacaacctctttttctgatcgggcctcggggctgtggtaaaacaacggtcggaatggcccttgccgattcgcttaaccgtcggtttgtcgataccgatcagtggttgcaatcacagctcaatatgacggtcgcggagatcgtcgaaagggaagagtgggcgggatttcgcgccagagaaacggcggcgctggaagcggtaactgcgccatccaccgttatcgctacaggcggcggcattattctgacggaatttaatcgtcacttcatgcaaaataacgggatcgtggtttatttgtgtgcgccagtatcagtcctggttaaccgactgcaagctgcaccggaagaagatttacggccaaccttaacgggaaaaccgctgagcgaagaagttcaggaagtgctggaagaacgcgatgcgctatatcgcgaagttgcgcatattatcatcgacgcaacaaacgaacccagccaggtgatttctgaaattcgcagcgccctggcacagacgatcaattgttgacaatctttagaggagacacaacatggtctttgtgtctgattcgtctatctctttgcccatttgggatgctccgcgcgctcgcggccccatagtctcggacctggctatccctggttccaagtcgatcaccaaccgcgccctcatcttggctgcgctcgcatcaactccatccaccatcattgatgtccttcgtagtcgtgataccgatctcatgactgatggtctacgcagcctcggaatcaccattactgaagaggcagtcgatcgctaccgcgttgagcccggacagttgtctgctggctccgttgagtgtggtcttgctggtacggtcatgcgctttttgcctcctgttgctgctttcgctgatggtcctgttcattttgatggcgatcctcaagctcgtgttcgtccgatgaccagcattttggatgcgctgcgttcgcttggtgtggaggtagacaacaacaatctgcctttcactgttaatgctggtgaggtccctgagggtggcgtggttgagattgatgcttccggctcatctcagtttgtttctggtcttttgctttcagcgcctcgttttaaaaatggcgtcaccgttaagcacgtcggtggtcgtctgccgagcatgccgcatattgagatgaccgtcgatatgcttcgttccgcaggcattgagatcgaagagtcagaaaatcagtgggttgttcatcctggtgagatcttgggtcggacctggcgcattgagccggatctttctaatgcgactccgttcctagctgccgctgcggtcactggtggaaccatcaagattaaccactggccaatcaaaactactcagcctggcgatgctattcgttcgattcttgagcgcatgggctgcgaagttgagctggttgctcagggtgaaggttacgatctgtcggtgactggtccggttgctctcaagggcattgagatcgatatgtccgatatcggtgagttgacccctaccgtggcggcgttggctgcgttggcgtcgacagagtctcgtttgaccggtattgctcatcttcgtggccatgagacggatcgtttggctgcgttgactgcggagatcaacaaacttggtggaaagtgcactgagcttaaggatggtctgttgattgagcctgcgtcgctgcacggtggtgtgtggcattcatatgctgatcaccgtatggctactgctggtgcgatcattggcctcgcggttgatggcgttcaggttgaagacattaagaccacttccaaaactttccctggttttgaaaatgtttgggaggagatggttggctaggcgaaagtcgtagccaccacgaagtccgaaaggaggcccttcagatgctaggcatgcttcgatggactacagcaggtgaatcccacggccaggcgcttatcgccacggttgaacacatgccagcaggcgtgcccgtgactaaagatgaggtctcgtatcaattggcgcgccgacgccttggatatggtcgcggcgctcgcatgaagtttgagcaagacgcgttgaccttcctcaccggcatccgccacggcctcactttgggtagccccatctcaatcatgatcggcaacactgagtgggataagtggaccaccatcatgtcctctgacgctttggacatggaagacccagataacgttgcggcgatgtcttcgggtcggggcgcaaaactgactcgtccgcgtccaggccacgctgattacgcaggcatgctcaagtacggattcgatgatgcccgcaacgtgctggagcgttcttcagcccgtgagacggcagcacgcgtggcagcagcaaccgttgcgcgttccttcctgcgtgaaaccttgggcgtggaagtgctttcccacgtaatttccattggtgcgtccgagccttacactggcgcggagccaacctttgcagatattcaagcaatcgatgattccccagttcgtgcattcggtaaagacgctgaagaatccatgatcgcggaaatcgaggccgcaaagaaagccggcgataccctcggtggcatcgtggaagtgattgttgaaggcctgcccatcggtttgggctcacacatttctggcgaagatcgcctcgatgcgcagatcgcagctgcactcatgggcattcaggccatcaagggcgtggaaatcggtgacggtttcgaagaagctcgtcgacgtggctccgaagcccacgatgaagtgttcctggatgacaacggcgtataccgcaacaccaaccgtgcaggtggcctcgaaggcggcatgaccaacggtgaaaccctgcgcgttcgtgctggcatgaagccaatttctactgtgcctcgcgccctgaaaaccattgatatggaaaacggcaaggcagcaaccggaatccaccagcgttccgacgtgtgcgctgttccagccgccggtgtcgttgcagaagcaatggtcaccctggttctcgcccgcgcagtcctgcagaaattcggcggtgactccctgagcgaaaccaagagcaacattgacacctacctcaaaaacattgaggaacgaatgaaattcgaaggtttagaggatggagcgtaa

SEQ ID NO: 16 - DNA, 3539 bp, artificial sequence
  Expressionskonstrukt
cacagggtagctggtagtttgaaaatcaacgccgttgcccttaggattcagtaactggcacattttgtaatgcgctagatctgtgtgctcagtcttccaggctgcttatcacagtgaaagcaaaaccaattcgtggctgcgaaagtcgtagccaccacgaagtccaggaggacatacatgaaaggaggcccttcagatgtccaacaccgtgttcatcggcgcaaaggaatacttcccaggcatcggcaagatcggcttcgaaggccgcgattccgataacccactggcattcaaggtgtacgatgcaaacaagcaggtggcaggcaagaccatggcagaacacctgcgcttcgcagtggcatactggcactccttctgcggcaacggcgcagatccattcggcccaggcacccgcgcatacccatgggatgtgggcaacaccgcactggcacgcgcagaagcaaagtccgatgcagcattcgaattcttcaccaagctgggcgtgccatactactgcttccacgatatcgatctggcaccagatgcagatgatatcggcgaatacgaaaacaacctgaagcacatggtgggcatcgcaaagcagcgccaggcagataccggcgtgaagctgctgtggggcaccgcaaacctgttctcccacccacgctacatgaacggcgcatccaccaacccagatttcaacgtggtggcacgcgcagcagtgcaggtgaaggcagcaatcgatgcaaccgtggaactgggcggcgaaaactacgtgttctggggcggccgcgaaggctacgcatgcctgcacaacacccagatgaagcgcgaacaggataacatggcacgcttcctgaccctggcacgcgattacggccgcgcaatcggcttcaccggcaacttcctgatcgaaccaaagccaatggaaccaatgaagcaccagtacgatttcgattccgcaaccgtgatcggcttcctgcgccagcacggcctggatcaggatttcaagctgaacatcgaagcaaaccacgcaaccctgtccggccactccttcgaacacgatctgcaggtggcatccgatgcaggcctgctgggctccatcgatgcaaaccgcggcaacccacagaacggctgggataccgatcagttcccaaccgatctgtacgataccgtgggcgcaatgctggtggtgctgcgccagggcggcctggcaccaggcggcctgaacttcgatgcaaaggtgcgccgcgaatcctccgatccacaggatctgttcctggcacacatcggcggcatggatgcattcgcacgcggcctggaagtggcaaacgcactgctgacctcctccccactggaaacctggcgcgcacagcgctacgcatccttcgattccggcgcaggcgcagatttcgcaaacggcacctccaccctggcagatctggcaaagtacgcagcaggcaagggcgaaccaacccaggtgtccggccgccaggaagcatacgaaaacctgatcaaccagtacctgacccgccacagggtagctggtagtttgaaaatcaacgccgttgcccttaggattcagtaactggcacattttgtaatgcgctagatctgtgtgctcagtcttccaggctgcttatcacagtgaaagcaaaaccaattcgtggctgcgaaagtcgtagccaccacgaagtccaggaggacatacatgaaaggaggcccttcagatggctttggttcttggaatcgatagttccacccaatcctgcaaggctttgcttgtcgatgccgccaccggccaggttatcgacgaaggccgcgcgagtcacccgagcgggtcggaggtagatccacgtgcgtggatcgctgcgctggatcaagctaccgaggggttgttagaacgcgcggacgctgtatctattgcaggccagcagcacggcatggtggcgttggatgaaaacgatgaaatcgttcgcccggcgttgttatggaatgacactcgttctgcccaggctgcgttggatctcaatgaggagatcggcggcgatcaggctgcggtagatgccacgggaagtgtgtatgttgcttctttaactgccaccaaaatgcggtggatgcgtgatcatgaaccagaaaatgcagcgcgcacggcgtcggtgatgttgcctcatgatttcctcacctggcatttgatgggacgcggacgcaaagtcaccgaccatggtgatgcttctggaacgggctactacagcacgcgtgatcgtgcgtggcgcaccgatctagctgccttggcgctgggccatgaggtggaacttcctgaactcctggccccaaatgcgattgcgggaacaactccaggtggagtgaaagttgctgcaggcacgggagataatgctgcggctgcgcttggccttgatttgcagcctggtgatgtcagcgtgtcgatcggcacctctggcgttgccggcatgaccgttcaacatagcgtccacgatccatctggtttggtcactggtttcgccgatgccacgggtgcgtatttcccgctggcctgcacgcttaatggcgcaccggtgttggaattcggccgccgcattctgggcgtggaatgggaagagttcgatgcgcttgcactggctgctcaacccggttcaggtggcgtgacgctccagccttatttggagggcgagcgtacgccgaatcgtcccgcagcacgtggcgttttggctggactaaactgtgcaacgacccgcgaggactttgcccgagcaactgttgaaggcttgttgttggcattggatgatgctgtaacggcgctggttgaggccacgggagtgcccgttcagcgcatccagctcatcggtggcggcgcgcgttcacaggcggttcgtgagattgcccctgagattttcggccatgagattgtggttccagaacccgctgaatatgtggcgttgggtgcagctcgtcaggcggcatgggcgctgtcgggtgaggccacgccaccgcagtggccaactcccggttccgatccgcaccgcgcacctaaaaacactgagctgagcacgcgttatgcgaagctgcgtgctgcaacgcagggttggtactagggctgttttggcggatgagagaagattttcagcctgatacagattaaatcagaacgcagaagcggtctgataaaacagaatttgcctggcggcagtagcgcggtggtcccacctgaccccatgccgaactcagaagtgaaacgccgtagcgccgatggtagtgtggggtctccccatgcgagagtagggaactgccaggcatcaaataaaacgaaaggctcagtcgaaagactgggcctttcgttttatctgttgtttgtcggtgaacgctctcctgagtaggacaaatccgccgggagcggatttgaacgttgcgaagcaacggcccggagggtggcgggcaggacgcccgccataaactgccaggcatcaaattaagcagaaggccatcctgacggatggcctttttgcgtttctacaaactct